European Patent Application EP 4 725 505 A1, published April 15, 2026. Title: Agent for prevent and/or treat of skin disorders associated with histone deacetylase 4 abnormality. Applicant: NATIONAL UNIVERSITY CORPORATION KOBE UNIVERSITY. The sequence listing filed with the application follows.

SEQUENCE LISTING (2 sequences)

SEQ ID NO: 1 - DNA, 16 bp, synthetic construct
  source 1..16: PCR_primers = fwd_seq: gctgtgtgcctaagtt,rev_seq:tgcaaaactaggaaaagttt; mol_type = other DNA
gctgtgtgcctaagtt

SEQ ID NO: 2 - DNA, 20 bp, synthetic construct
  source 1..20: PCR_primers = fwd_seq: gctgtgtgcctaagtt,rev_seq:tgcaaaactaggaaaagttt; mol_type = other DNA
tgcaaaactaggaaaagttt